European Patent Application EP 4 549 938 A1, published May 7, 2025. Title: 血管炎への罹患状態またはＣＯＶＩＤ－１９の重症化リスクを検査する方法、検査用キット、コンパニオン診断薬、および検査用マーカー. Applicant: 国立大学法人千葉大学. The sequence listing filed with the application follows.

SEQUENCE LISTING (2 sequences)

SEQ ID NO: 1 - protein, 265 aa, synthetic construct
  REGION 1..265: note = Amino acid sequence of VasSF antibody
MDFGLSWIFLVALLRGVQCQVHLVESGGGLVQPGRSLRLSCAVSGFTFASYAMHWVRQAPGKGLEWVAGISKDGSNKRHADSLEGRFTISRDNSKNTLYLQVSGLRAEDTAVYYCARSQDPTDFDWLLSEHWGQGTLVTVSSASTKGPSVFPLAPCSRSTSESTAALGCLVKDYFPEPVTVSWNSGALTSGVHTFPAVLQSSGLYSLSSVVTVPSSNFGTQTYTCNVDHKPSNTKVDKTVAPPVAGPSVFLFPPKPKDTHHHHHH

SEQ ID NO: 2 - DNA, 798 bp, synthetic construct
  misc_feature 1..798: note = DNA sequence coding VasSF antibody
  source 1..798: mol_type = other DNA
atggatttcggccttagctggattttcctggtagcgctgctgcgtggcgtacagtgccaagtacacttagtggagtctggtggtggcttggttcaaccgggtcgttctctgcggctctcatgtgcggtgagcggcttcacctttgcgtcctatgccatgcattgggtccgtcaggctcctggcaaagggctggaatgggtcgcagggatcagtaaggatgggagcaacaaacgtcatgccgatagcctcgaaggccgctttaccattagtcgcgataactcgaagaacaccctgtatctccaggttagtggcttacgcgcagaagataccgccgtttactattgtgcgcgctcacaagatccgacggacttcgattggcttctgtccgaacattggggtcagggtactctggtgacagtctcgtcagcgagcacaaaaggcccgtcggtgtttccgttagccccttgttctcgcagtacttccgagagtactgctgcactgggttgcctggtgaaagactacttcccggaaccggttaccgtgtcgtggaattcaggtgcactgacctctggagtccatacgtttcctgcggttttgcagtcgagcggcttgtactctctgagcagcgttgtgacggtgccgagctccaactttggaacccagacctatacgtgcaatgtggatcacaaaccctccaatacgaaggtagacaaaaccgtggctccaccagttgccggtccaagcgtctttctgtttccgcccaaaccgaaagacacacatcaccaccatcaccattaa